European Patent Application EP 4 230 643 A1, published August 23, 2023. Title: Polypeptide, polymer, solid phase, a method for measuring a target substance and  a reagent kit therefor. Applicant: SYSMEX CORPORATION. The sequence listing filed with the application follows.

SEQUENCE LISTING (9 sequences)

SEQ ID NO: 1 - protein, 159 aa, Streptomyces avidinii
DPSKDSKAQVSAAEAGITGTWYNQLGSTFIVTAGADGALTGTYESAVGNAESRYVLTGRYDSAPATDGSGTALGWTVAWKNNYRNAHSATTWSGQYVGGAEARINTQWLLTSGTTEANAWKSTLVGHDTFTKVKPSAASIDAAKKAGVNNGNPLDAVQQ

SEQ ID NO: 2 - protein, 128 aa, Gallus gallus
ARKCSLTGKWTNDLGSNMTIGAVNSRGEFTGTYITAVTATSNEIKESPLHGTQNTINKRTQPTFGFTVNWKFSESTTVFTGQCFIDRNGKEVLKTMWLLRSSVNDIGDDWKATRVGINIFTRLRTQKE

SEQ ID NO: 3 - protein, 143 aa, Pleurotus cornucopiae
MKDVQSLLTGTWYNELGSTMNLTANKDGSLTGTYHSNVGEVPPTYHLSGRYNLQPPSGQGVTLGWAVSFENTSANVHSVSTWSGQYFSEPAEVILTQWLLSRSSEREDLWQSTHVGHDEFSKTKPTKEKIAQAQLLRRGLKFE

SEQ ID NO: 4 - protein, 141 aa, Pleurotus cornucopiae
MSDVQSSLTGTWYNELNSKMELTANKDGTLTGKYLSKVGDVYVPYPLSGRYNLQPPAGQGVALGWAVSWENSKIHSATTWSGQFFSESSPVILTQWLLSSSTARGDVWESTLVGNDSFTKTAPTEQQIAHAQLHCRAPRLK

SEQ ID NO: 5 - protein, 159 aa, Artificial Sequence
  Comprising modified amino acid sequence.
DPSKDSKAQVSAAEAGITGTWYNQLGSTFIVTAGADGALTGTYEAAVGNAESRYVLTGRYDSAPATDGSGTALGWTVAWKNNYRNAHSAATWSGQYVGGAEARINTQWLLTSGTTEANAWKSTLVGHATFTKVKPSAASIDAAKKAGVNNGNPLDAVQQ

SEQ ID NO: 6 - protein, 159 aa, Artificial Sequence
  Comprising modified amino acid sequence.
DPSKDSKAQVSAAEAGITGTWYNQLGSTFIVTAGADGALTGTYESAVGNAESRYTLTGRYDSAPARDGSGTALGWTVAWKNNYRNAHSATTWSGQYVGGAEARINTQWTLTSGTTEANAWKSTLRGHDTFTKVKPSAASIDAAKKAGVNNGNPLDAVQQ

SEQ ID NO: 7 - protein, 114 aa, Artificial Sequence
  Comprising modified amino acid sequence.
AEAGITGTWYNQSGSTFTVTAGADGNLTGQYENRAQGTGCQNSPYTLTGRYNGTKLEWRVEWNNSTENCHSRTEWRGQYQGGAEARINTQWNLTYEGGSGPATEQGQDTFTKVK

SEQ ID NO: 8 - protein, 151 aa, Artificial Sequence
  Comprising modified amino acid sequence.
DPSKDSKAQVSAAEAGITGTWYNQLGSTFIVTAGADGALTGTYESAVGNAESRYVLTGRYDSAPATDGSGTALGWTVAWKNNYRNAHSATTWSGQYVGGAEARINTQWLLTSKSTLVGDDTFTKVKPSAASIDAAKKAGVNNGNPLDAVQQ

SEQ ID NO: 9 - protein, 273 aa, Artificial Sequence
  Comprising modified amino acid sequence.
EANAKKSTLVGHDTFTKVKPSAASGGGSAEAGITGTWYNQLGSTFIVTAGADGALTGTYESAVGNAESRYVLTGRYDSAPATDGSGTALGWTVAWKNNYRNAHSATTWSGQYVGGAEARINTQWLLTSGTGSGTALGWTVAWKNNYRNAHSATTWSGQYVGGAEARINTQWLLTSGTTEANAWKSTLVGHDTFTKVKPSAASGGGSAEVGITGTWYNQLGSTFIVTAGADGALTGTYESAVGNAESRYVLTGRYDSAPATDGAAALEHHHHHH